European Patent Application EP 4 548 757 A1, published May 7, 2025. Title: Method for producing nonhuman primate animal model of cerebral infarction and pharmaceutical composition for treatment of cerebral infarction. Applicant: アステラス製薬株式会社. The sequence listing filed with the application follows.

SEQUENCE LISTING (14 sequences)

SEQ ID NO: 1 - DNA, 5015 bp, synthetic construct
  misc_feature 1..5015: note = NeuroD1-expressing vector AAV-GFAP-Neurod1-IRES-GFP
  source 1..5015: mol_type = other DNA
tacgaattgcctgcaggcagctgcgcgctcgctcgctcactgaggccgcccgggcaaagcccgggcgtcgggcgacctttggtcgcccggcctcagtgagcgagcgagcgcgcagagagggagtggccaactccatcactaggggttcctatcgatatcaagctttaatagtctgcaagcagacctggcagcattgggctggccgccccccagggcctcctcttcatgcccagtgaatgactcaccttggcacagacacaatgttcggggtgggcacagtgcctgcttcccgccgcaccccagcccccctcaaatgccttccgagaagcccattgagtagggggcttgcattgcaccccagcctgacagcctggcatcttgggataaaagcagcacagccccctaggggctgcccttgctgtgtggcgccaccggcggtggagaacaaggctctattcagcctgtgcccaggaaaggggatcaggggatgcccaggcatggacagtgggtggcagggggggagaggagggctgtctgcttcccagaagtccaaggacacaaatgggtgaggggactgggcagggttctgaccctgtgggaccagagtggagggcgtagatggacctgaagtctccagggacaacagggcccaggtctcaggctcctagttgggcccagtggctccagcgtttccaaacccatccatccccagaggttcttcccatctctccaggctgatgtgtgggaactcgaggaaataaatctccagtgggagacggaggggtggccagggaaacggggcgctgcaggaataaagacgagccagcacagccagctcatgcgtaacggctttgtggagctgtcaaggcctggtctctgggagagaggcacagggaggccagacaaggaaggggtgacctggagggacagatccaggggctaaagtcctgataaggcaagagagtgccggccccctcttgccctatcaggacctccactgccacatagaggccatgattgacccttagacaaagggctggtgtccaatcccagcccccagccccagaactccagggaatgaatgggcagagagcaggaatgtgggacatctgtgttcaagggaaggactccaggagtctgctgggaatgaggcctagtaggaaatgaggtggcccttgagggtacagaacaggttcattcttcgccaaattcccagcaccttgcaggcacttacagctgagtgagataatgcctgggttatgaaatcaaaaagttggaaagcaggtcagaggtcatctggtacagcccttccttccctttttttttttttttttttgtgagacaaggtctctctctgttgcccaggctggagtggcgcaaacacagctcactgcagcctcaacctactgggctcaagcaatcctccagcctcagcctcccaaagtgctgggattacaagcatgagccaccccactcagccctttccttcctttttaattgatgcataataattgtaagtattcatcatggtccaaccaaccctttcttgacccaccttcctagagagagggtcctcttgattcagcggtcagggccccagacccatggtctggctccaggtaccacctgcctcatgcaggagttggcgtgcccaggaagctctgcctctgggcacagtgacctcagtggggtgaggggagctctccccatagctgggctgcggcccaaccccaccccctcaggctatgccagggggtgttgccaggggcacccgggcatcgccagtctagcccactccttcataaagccctcgcatcccaggagcgagcagagccagagcatcgaatcccggccgggaacggtgcattggaacgcggattccccgtgccaagagtgacgtaagtaccgcctatagagtctataggcccacaaaaaatgctttcttcttttaatatacttttttgtttatcttatttctaatactttccctaatctctttctttcagggcaataatgatacaatgtatcatgcctctttgcaccattctaaagaataacagtgataatttctgggttaaggcaatagcaatatttctgcatataaatatttctgcatataaattgtaactgatgtaagaggtttcatattgctaatagcagctacaatccagctaccattctgcttttattttatggttgggataaggctggattattctgagtccaagctaggcccttttgctaatcatgttcatacctcttatcttcctcccacagctcctgggcaacgtgctggtctgtgtgctggcccatcactttggcaaagaattgggattcgcgagaattctgccaccatgaccaaatcatacagcgagagcgggctgatgggcgagcctcagccccaaggtcccccaagctggacagatgagtgtctcagttctcaggacgaggaacacgaggcagacaagaaagaggacgagcttgaagccatgaatgcagaggaggactctctgagaaacgggggagaggaggaggaggaagatgaggatctagaggaagaggaggaagaagaagaggaggaggaggatcaaaagcccaagagacggggtcccaaaaagaaaaagatgaccaaggcgcgcctagaacgttttaaattaaggcgcatgaaggccaacgcccgcgagcggaaccgcatgcacgggctgaacgcggcgctggacaacctgcgcaaggtggtaccttgctactccaagacccagaaactgtctaaaatagagacactgcgcttggccaagaactacatctgggctctgtcagagatcctgcgctcaggcaaaagccctgatctggtctccttcgtacagacgctctgcaaaggtttgtcccagcccactaccaatttggtcgccggctgcctgcagctcaaccctcggactttcttgcctgagcagaacccggacatgcccccgcatctgccaaccgccagcgcttccttcccggtgcatccctactcctaccagtcccctggactgcccagcccgccctacggcaccatggacagctcccacgtcttccacgtcaagccgccgccacacgcctacagcgcagctctggagcccttctttgaaagccccctaactgactgcaccagcccttcctttgacggacccctcagcccgccgctcagcatcaatggcaacttctctttcaaacacgaaccatccgccgagtttgaaaaaaattatgcctttaccatgcactaccctgcagcgacgctggcagggccccaaagccacggatcaatcttctcttccggtgccgctgcccctcgctgcgagatccccatagacaacattatgtctttcgatagccattcgcatcatgagcgagtcatgagtgcccagcttaatgccatctttcacgattaggtttaaacgcggccgcgcccctctccctcccccccccctaacgttactggccgaagccgcttggaataaggccggtgtgcgtttgtctatatgttattttccaccatattgccgtcttttggcaatgtgagggcccggaaacctggccctgtcttcttgacgagcattcctaggggtctttcccctctcgccaaaggaatgcaaggtctgttgaatgtcgtgaaggaagcagttcctctggaagcttcttgaagacaaacaacgtctgtagcgaccctttgcaggcagcggaaccccccacctggcgacaggtgcctctgcggccaaaagccacgtgtataagatacacctgcaaaggcggcacaaccccagtgccacgttgtgagttggatagttgtggaaagagtcaaatggctctcctcaagcgtattcaacaaggggctgaaggatgcccagaaggtaccccattgtatgggatctgatctggggcctcggtgcacatgctttacatgtgtttagtcgaggttaaaaaaacgtctaggccccccgaaccacggggacgtggttttcctttgaaaaacacgatgataatatggccacaaccatggtgagcaagggcgaggagctgttcaccggggtggtgcccatcctggtcgagctggacggcgacgtaaacggccacaagttcagcgtgtccggcgagggcgagggcgatgccacctacggcaagctgaccctgaagttcatctgcaccaccggcaagctgcccgtgccctggcccaccctcgtgaccaccctgacctacggcgtgcagtgcttcagccgctaccccgaccacatgaagcagcacgacttcttcaagtccgccatgcccgaaggctacgtccaggagcgcaccatcttcttcaaggacgacggcaactacaagacccgcgccgaggtgaagttcgagggcgacaccctggtgaaccgcatcgagctgaagggcatcgacttcaaggaggacggcaacatcctggggcacaagctggagtacaactacaacagccacaacgtctatatcatggccgacaagcagaagaacggcatcaaggtgaacttcaagatccgccacaacatcgaggacggcagcgtgcagctcgccgaccactaccagcagaacacccccatcggcgacggccccgtgctgctgcccgacaaccactacctgagcacccagtccgccctgagcaaagaccccaacgagaagcgcgatcacatggtcctgctggagttcgtgaccgccgccgggatcactctcggcatggacgagctgtacaagtaaatagatctaggaacccctagtgatggagttggccactccctctctgcgcgctcgctcgctcactgaggccgggcgaccaaaggtcgcccgacgcccgggctttgcccgggcggcctcagtgagcgagcgagcgcgcagctgcctgcaggcagcttggcactggccgtcgttttacaacgtcgtgactgggaaaaccctggcgttacccaacttaatcgccttgcagcacatccccctttcgccagctggcgtaatagcgaaga

SEQ ID NO: 2 - DNA, 3401 bp, synthetic construct
  misc_feature 1..3401: note = Control vector AAV-GFAP-GFP
  source 1..3401: mol_type = other DNA
gattacgaattgcctgcaggcagctgcgcgctcgctcgctcactgaggccgcccgggcaaagcccgggcgtcgggcgacctttggtcgcccggcctcagtgagcgagcgagcgcgcagagagggagtggccaactccatcactaggggttcctatcgatatcaagctttaatagtctgcaagcagacctggcagcattgggctggccgccccccagggcctcctcttcatgcccagtgaatgactcaccttggcacagacacaatgttcggggtgggcacagtgcctgcttcccgccgcaccccagcccccctcaaatgccttccgagaagcccattgagtagggggcttgcattgcaccccagcctgacagcctggcatcttgggataaaagcagcacagccccctaggggctgcccttgctgtgtggcgccaccggcggtggagaacaaggctctattcagcctgtgcccaggaaaggggatcaggggatgcccaggcatggacagtgggtggcagggggggagaggagggctgtctgcttcccagaagtccaaggacacaaatgggtgaggggactgggcagggttctgaccctgtgggaccagagtggagggcgtagatggacctgaagtctccagggacaacagggcccaggtctcaggctcctagttgggcccagtggctccagcgtttccaaacccatccatccccagaggttcttcccatctctccaggctgatgtgtgggaactcgaggaaataaatctccagtgggagacggaggggtggccagggaaacggggcgctgcaggaataaagacgagccagcacagccagctcatgcgtaacggctttgtggagctgtcaaggcctggtctctgggagagaggcacagggaggccagacaaggaaggggtgacctggagggacagatccaggggctaaagtcctgataaggcaagagagtgccggccccctcttgccctatcaggacctccactgccacatagaggccatgattgacccttagacaaagggctggtgtccaatcccagcccccagccccagaactccagggaatgaatgggcagagagcaggaatgtgggacatctgtgttcaagggaaggactccaggagtctgctgggaatgaggcctagtaggaaatgaggtggcccttgagggtacagaacaggttcattcttcgccaaattcccagcaccttgcaggcacttacagctgagtgagataatgcctgggttatgaaatcaaaaagttggaaagcaggtcagaggtcatctggtacagcccttccttccctttttttttttttttttttgtgagacaaggtctctctctgttgcccaggctggagtggcgcaaacacagctcactgcagcctcaacctactgggctcaagcaatcctccagcctcagcctcccaaagtgctgggattacaagcatgagccaccccactcagccctttccttcctttttaattgatgcataataattgtaagtattcatcatggtccaaccaaccctttcttgacccaccttcctagagagagggtcctcttgattcagcggtcagggccccagacccatggtctggctccaggtaccacctgcctcatgcaggagttggcgtgcccaggaagctctgcctctgggcacagtgacctcagtggggtgaggggagctctccccatagctgggctgcggcccaaccccaccccctcaggctatgccagggggtgttgccaggggcacccgggcatcgccagtctagcccactccttcataaagccctcgcatcccaggagcgagcagagccagagcatcgaatcccggccgggaacggtgcattggaacgcggattccccgtgccaagagtgacgtaagtaccgcctatagagtctataggcccacaaaaaatgctttcttcttttaatatacttttttgtttatcttatttctaatactttccctaatctctttctttcagggcaataatgatacaatgtatcatgcctctttgcaccattctaaagaataacagtgataatttctgggttaaggcaatagcaatatttctgcatataaatatttctgcatataaattgtaactgatgtaagaggtttcatattgctaatagcagctacaatccagctaccattctgcttttattttatggttgggataaggctggattattctgagtccaagctaggcccttttgctaatcatgttcatacctcttatcttcctcccacagctcctgggcaacgtgctggtctgtgtgctggcccatcactttggcaaagaattgggattcgcgagaattctgccaccatggtgagcaagggcgaggagctgttcaccggggtggtgcccatcctggtcgagctggacggcgacgtaaacggccacaagttcagcgtgtccggcgagggcgagggcgatgccacctacggcaagctgaccctgaagttcatctgcaccaccggcaagctgcccgtgccctggcccaccctcgtgaccaccctgacctacggcgtgcagtgcttcagccgctaccccgaccacatgaagcagcacgacttcttcaagtccgccatgcccgaaggctacgtccaggagcgcaccatcttcttcaaggacgacggcaactacaagacccgcgccgaggtgaagttcgagggcgacaccctggtgaaccgcatcgagctgaagggcatcgacttcaaggaggacggcaacatcctggggcacaagctggagtacaactacaacagccacaacgtctatatcatggccgacaagcagaagaacggcatcaaggtgaacttcaagatccgccacaacatcgaggacggcagcgtgcagctcgccgaccactaccagcagaacacccccatcggcgacggccccgtgctgctgcccgacaaccactacctgagcacccagtccgccctgagcaaagaccccaacgagaagcgcgatcacatggtcctgctggagttcgtgaccgccgccgggatcactctcggcatggacgagctgtacaagtaaatagatctaggaacccctagtgatggagttggccactccctctctgcgcgctcgctcgctcactgaggccgggcgaccaaaggtcgcccgacgcccgggctttgcccgggcggcctcagtgagcgagcgagcgcgcagctgcctgcaggcagcttggcactggccgtcgttttacaacgtcgtgactgggaaaaccctggcgttacccaacttaatcgccttgcagcacatccccctttcgccagctggcgtaatagcgaagaggcccgcaccgatcgcccttcccaacagttgcgcagcctgaatggcgaatggcgcctgatg

SEQ ID NO: 3 - DNA, 720 bp, unidentified
  misc_feature 1..720: note = GFP gene (CDS)
  source 1..720: mol_type = genomic DNA
  CDS 1..720: protein_id = 4; translation = MVSKGEELFTGVVPILVELDGDVNGHKFSVSGEGEGDATYGKLTLKFICTTGKLPVPWPTLVTTLTYGVQCFSRYPDHMKQHDFFKSAMPEGYVQERTIFFKDDGNYKTRAEVKFEGDTLVNRIELKGIDFKEDGNILGHKLEYNYNSHNVYIMADKQKNGIKVNFKIRHNIEDGSVQLADHYQQNTPIGDGPVLLPDNHYLSTQSALSKDPNEKRDHMVLLEFVTAAGITLGMDELYK
atggtgagcaagggcgaggagctgttcaccggggtggtgcccatcctggtcgagctggacggcgacgtaaacggccacaagttcagcgtgtccggcgagggcgagggcgatgccacctacggcaagctgaccctgaagttcatctgcaccaccggcaagctgcccgtgccctggcccaccctcgtgaccaccctgacctacggcgtgcagtgcttcagccgctaccccgaccacatgaagcagcacgacttcttcaagtccgccatgcccgaaggctacgtccaggagcgcaccatcttcttcaaggacgacggcaactacaagacccgcgccgaggtgaagttcgagggcgacaccctggtgaaccgcatcgagctgaagggcatcgacttcaaggaggacggcaacatcctggggcacaagctggagtacaactacaacagccacaacgtctatatcatggccgacaagcagaagaacggcatcaaggtgaacttcaagatccgccacaacatcgaggacggcagcgtgcagctcgccgaccactaccagcagaacacccccatcggcgacggccccgtgctgctgcccgacaaccactacctgagcacccagtccgccctgagcaaagaccccaacgagaagcgcgatcacatggtcctgctggagttcgtgaccgccgccgggatcactctcggcatggacgagctgtacaagtaa

SEQ ID NO: 4 - protein, 239 aa, unidentified
  REGION 1..239: note = GFP
MVSKGEELFTGVVPILVELDGDVNGHKFSVSGEGEGDATYGKLTLKFICTTGKLPVPWPTLVTTLTYGVQCFSRYPDHMKQHDFFKSAMPEGYVQERTIFFKDDGNYKTRAEVKFEGDTLVNRIELKGIDFKEDGNILGHKLEYNYNSHNVYIMADKQKNGIKVNFKIRHNIEDGSVQLADHYQQNTPIGDGPVLLPDNHYLSTQSALSKDPNEKRDHMVLLEFVTAAGITLGMDELYK

SEQ ID NO: 5 - DNA, 1074 bp, Mus musculus
  misc_feature 1..1074: note = mouse NeuroD1 gene (CDS)
  source 1..1074: mol_type = genomic DNA
  CDS 1..1074: protein_id = 6; translation = MTKSYSESGLMGEPQPQGPPSWTDECLSSQDEEHEADKKEDELEAMNAEEDSLRNGGEEEEEDEDLEEEEEEEEEEEDQKPKRRGPKKKKMTKARLERFKLRRMKANARERNRMHGLNAALDNLRKVVPCYSKTQKLSKIETLRLAKNYIWALSEILRSGKSPDLVSFVQTLCKGLSQPTTNLVAGCLQLNPRTFLPEQNPDMPPHLPTASASFPVHPYSYQSPGLPSPPYGTMDSSHVFHVKPPPHAYSAALEPFFESPLTDCTSPSFDGPLSPPLSINGNFSFKHEPSAEFEKNYAFTMHYPAATLAGPQSHGSIFSSGAAAPRCEIPIDNIMSFDSHSHHERVMSAQLNAIFHD
atgaccaaatcatacagcgagagcgggctgatgggcgagcctcagccccaaggtcccccaagctggacagatgagtgtctcagttctcaggacgaggaacacgaggcagacaagaaagaggacgagcttgaagccatgaatgcagaggaggactctctgagaaacgggggagaggaggaggaggaagatgaggatctagaggaagaggaggaagaagaagaggaggaggaggatcaaaagcccaagagacggggtcccaaaaagaaaaagatgaccaaggcgcgcctagaacgttttaaattaaggcgcatgaaggccaacgcccgcgagcggaaccgcatgcacgggctgaacgcggcgctggacaacctgcgcaaggtggtaccttgctactccaagacccagaaactgtctaaaatagagacactgcgcttggccaagaactacatctgggctctgtcagagatcctgcgctcaggcaaaagccctgatctggtctccttcgtacagacgctctgcaaaggtttgtcccagcccactaccaatttggtcgccggctgcctgcagctcaaccctcggactttcttgcctgagcagaacccggacatgcccccgcatctgccaaccgccagcgcttccttcccggtgcatccctactcctaccagtcccctggactgcccagcccgccctacggcaccatggacagctcccacgtcttccacgtcaagccgccgccacacgcctacagcgcagctctggagcccttctttgaaagccccctaactgactgcaccagcccttcctttgacggacccctcagcccgccgctcagcatcaatggcaacttctctttcaaacacgaaccatccgccgagtttgaaaaaaattatgcctttaccatgcactaccctgcagcgacgctggcagggccccaaagccacggatcaatcttctcttccggtgccgctgcccctcgctgcgagatccccatagacaacattatgtctttcgatagccattcgcatcatgagcgagtcatgagtgcccagcttaatgccatctttcacgattag

SEQ ID NO: 6 - protein, 357 aa, Mus musculus
  REGION 1..357: note = mouse NeuroD1 protein
MTKSYSESGLMGEPQPQGPPSWTDECLSSQDEEHEADKKEDELEAMNAEEDSLRNGGEEEEEDEDLEEEEEEEEEEEDQKPKRRGPKKKKMTKARLERFKLRRMKANARERNRMHGLNAALDNLRKVVPCYSKTQKLSKIETLRLAKNYIWALSEILRSGKSPDLVSFVQTLCKGLSQPTTNLVAGCLQLNPRTFLPEQNPDMPPHLPTASASFPVHPYSYQSPGLPSPPYGTMDSSHVFHVKPPPHAYSAALEPFFESPLTDCTSPSFDGPLSPPLSINGNFSFKHEPSAEFEKNYAFTMHYPAATLAGPQSHGSIFSSGAAAPRCEIPIDNIMSFDSHSHHERVMSAQLNAIFHD

SEQ ID NO: 7 - DNA, 1071 bp, Homo sapiens
  misc_feature 1..1071: note = human NeuroD1 gene (CDS)
  source 1..1071: mol_type = genomic DNA
  CDS 1..1071: protein_id = 8; translation = MTKSYSESGLMGEPQPQGPPSWTDECLSSQDEEHEADKKEDDLETMNAEEDSLRNGGEEEDEDEDLEEEEEEEEEDDDQKPKRRGPKKKKMTKARLERFKLRRMKANARERNRMHGLNAALDNLRKVVPCYSKTQKLSKIETLRLAKNYIWALSEILRSGKSPDLVSFVQTLCKGLSQPTTNLVAGCLQLNPRTFLPEQNQDMPPHLPTASASFPVHPYSYQSPGLPSPPYGTMDSSHVFHVKPPPHAYSAALEPFFESPLTDCTSPSFDGPLSPPLSINGNFSFKHEPSAEFEKNYAFTMHYPAATLAGAQSHGSIFSGTAAPRCEIPIDNIMSFDSHSHHERVMSAQLNAIFHD
atgaccaaatcgtacagcgagagtgggctgatgggcgagcctcagccccaaggtcctccaagctggacagacgagtgtctcagttctcaggacgaggagcacgaggcagacaagaaggaggacgacctcgaaaccatgaacgcagaggaggactcactgaggaacgggggagaggaggaggacgaagatgaggacctggaagaggaggaagaagaggaagaggaggatgacgatcaaaagcccaagagacgcggccccaaaaagaagaagatgactaaggctcgcctggagcgttttaaattgagacgcatgaaggctaacgcccgggagcggaaccgcatgcacggactgaacgcggcgctagacaacctgcgcaaggtggtgccttgctattctaagacgcagaagctgtccaaaatcgagactctgcgcttggccaagaactacatctgggctctgtcggagatcctgcgctcaggcaaaagcccagacctggtctccttcgttcagacgctttgcaagggcttatcccaacccaccaccaacctggttgcgggctgcctgcaactcaatcctcggacttttctgcctgagcagaaccaggacatgcccccccacctgccgacggccagcgcttccttccctgtacacccctactcctaccagtcgcctgggctgcccagtccgccttacggtaccatggacagctcccatgtcttccacgttaagcctccgccgcacgcctacagcgcagcgctggagcccttctttgaaagccctctgactgattgcaccagcccttcctttgatggacccctcagcccgccgctcagcatcaatggcaacttctctttcaaacacgaaccgtccgccgagtttgagaaaaattatgcctttaccatgcactatcctgcagcgacactggcaggggcccaaagccacggatcaatcttctcaggcaccgctgcccctcgctgcgagatccccatagacaatattatgtccttcgatagccattcacatcatgagcgagtcatgagtgcccagctcaatgccatatttcatgattag

SEQ ID NO: 8 - protein, 356 aa, Homo sapiens
  REGION 1..356: note = human NeuroD1 protein
MTKSYSESGLMGEPQPQGPPSWTDECLSSQDEEHEADKKEDDLETMNAEEDSLRNGGEEEDEDEDLEEEEEEEEEDDDQKPKRRGPKKKKMTKARLERFKLRRMKANARERNRMHGLNAALDNLRKVVPCYSKTQKLSKIETLRLAKNYIWALSEILRSGKSPDLVSFVQTLCKGLSQPTTNLVAGCLQLNPRTFLPEQNQDMPPHLPTASASFPVHPYSYQSPGLPSPPYGTMDSSHVFHVKPPPHAYSAALEPFFESPLTDCTSPSFDGPLSPPLSINGNFSFKHEPSAEFEKNYAFTMHYPAATLAGAQSHGSIFSGTAAPRCEIPIDNIMSFDSHSHHERVMSAQLNAIFHD

SEQ ID NO: 9 - protein, 21 aa, Homo sapiens
  REGION 1..21: note = endothelin-1 (human-derived)
CSCSSLMDKECVYFCHLDIIW

SEQ ID NO: 10 - DNA, 1071 bp, Homo sapiens
  source 1..1071: mol_type = genomic DNA
  CDS 1..1071: protein_id = 8; translation = MTKSYSESGLMGEPQPQGPPSWTDECLSSQDEEHEADKKEDDLETMNAEEDSLRNGGEEEDEDEDLEEEEEEEEEDDDQKPKRRGPKKKKMTKARLERFKLRRMKANARERNRMHGLNAALDNLRKVVPCYSKTQKLSKIETLRLAKNYIWALSEILRSGKSPDLVSFVQTLCKGLSQPTTNLVAGCLQLNPRTFLPEQNQDMPPHLPTASASFPVHPYSYQSPGLPSPPYGTMDSSHVFHVKPPPHAYSAALEPFFESPLTDCTSPSFDGPLSPPLSINGNFSFKHEPSAEFEKNYAFTMHYPAATLAGAQSHGSIFSGTAAPRCEIPIDNIMSFDSHSHHERVMSAQLNAIFHD
  misc_feature 1..1071: note = human NeuroD1 gene (CDS)
atgaccaaatcgtacagcgagagtgggctgatgggcgagcctcagccccaaggtcctccaagctggacagacgagtgtctcagttctcaggacgaggagcacgaggcagacaagaaggaggacgacctcgaaaccatgaacgcagaggaggactcactgaggaacgggggagaggaggaggacgaagatgaggacctggaagaggaggaagaagaggaagaggaggatgacgatcaaaagcccaagagacgcggccccaaaaagaagaagatgactaaggctcgcctggagcgttttaaattgagacgcatgaaggctaacgcccgggagcggaaccgcatgcacggactgaacgcggcgctagacaacctgcgcaaggtggtgccttgctattctaagacgcagaagctgtccaaaatcgagactctgcgcttggccaagaactacatctgggctctgtcggagatcctgcgctcaggcaaaagcccagacctggtctccttcgttcagacgctttgcaagggcttatcccaacccaccaccaacctggttgcgggctgcctgcaactcaatcctcggacttttctgcctgagcagaaccaggacatgcccccccacctgccgacggccagcgcttccttccctgtacacccctactcctaccagtcgcctgggctgcccagtccgccttacggtaccatggacagctcccatgtcttccacgttaagcctccgccgcacgcctacagcgcagcgctggagcccttctttgaaagccctctgactgattgcaccagcccttcctttgatggacccctcagcccgccgctcagcatcaatggcaacttctctttcaaacacgaaccgtccgccgagtttgagaaaaattatgcctttaccatgcactatcctgcagcgacactggcaggggcccaaagccacggatcaatcttctcaggcaccgctgcccctcgctgcgagatccccatagacaatattatgtccttcgatagccattcacatcatgagcgagtcatgagtgcccagctcaatgccatatttcatgattaa

SEQ ID NO: 11 - RNA, 1310 nt, Homo sapiens
  source 1..1310: mol_type = mRNA
  misc_feature 1..1310: note = human NeuroD1 mRNA sequence (ND1-2)
aggactcttctggtccccacagactcagagagaacccgccaccatgaccaaatcgtacagcgagagtgggctgatgggcgagcctcagccccaaggtcctccaagctggacagacgagtgtctcagttctcaggacgaggagcacgaggcagacaagaaggaggacgacctcgaaaccatgaacgcagaggaggactcactgaggaacgggggagaggaggaggacgaagatgaggacctggaagaggaggaagaagaggaagaggaggatgacgatcaaaagcccaagagacgcggccccaaaaagaagaagatgactaaggctcgcctggagcgttttaaattgagacgcatgaaggctaacgcccgggagcggaaccgcatgcacggactgaacgcggcgctagacaacctgcgcaaggtggtgccttgctattctaagacgcagaagctgtccaaaatcgagactctgcgcttggccaagaactacatctgggctctgtcggagatcctgcgctcaggcaaaagcccagacctggtctccttcgttcagacgctttgcaagggcttatcccaacccaccaccaacctggttgcgggctgcctgcaactcaatcctcggacttttctgcctgagcagaaccaggacatgcccccccacctgccgacggccagcgcttccttccctgtacacccctactcctaccagtcgcctgggctgcccagtccgccttacggtaccatggacagctcccatgtcttccacgttaagcctccgccgcacgcctacagcgcagcgctggagcccttctttgaaagccctctgactgattgcaccagcccttcctttgatggacccctcagcccgccgctcagcatcaatggcaacttctctttcaaacacgaaccgtccgccgagtttgagaaaaattatgcctttaccatgcactatcctgcagcgacactggcaggggcccaaagccacggatcaatcttctcaggcaccgctgcccctcgctgcgagatccccatagacaatattatgtccttcgatagccattcacatcatgagcgagtcatgagtgcccagctcaatgccatatttcatgattaatgataggctggagcctcggtggccatgcttcttgccccttgggcctccccccagcccctcctccccttcctgcacccgtacccccgtggtctttgaataaagtctgagtgggcggcaaaaaaaaaaaaaaaaaaaaaaaaaaaaaaaaaaaaaaaaaaaaaaaaaaaaaaaaaaaaaaaaaaaaaaaaaaaaaaaa

SEQ ID NO: 12 - DNA, 8192 bp, synthetic construct
  source 1..8192: mol_type = other DNA
  misc_feature 1..8192: note = pRC_AAV9
gcgcgccgatatcgttaacgccccgcgccggccgctctagaactagtggatcccccggaagatcagaagttcctattccgaagttcctattctctagaaagtataggaacttctgatctgcgcagccgccatgccggggttttacgagattgtgattaaggtccccagcgaccttgacgagcatctgcccggcatttctgacagctttgtgaactgggtggccgagaaggaatgggagttgccgccagattctgacatggatctgaatctgattgagcaggcacccctgaccgtggccgagaagctgcagcgcgactttctgacggaatggcgccgtgtgagtaaggccccggaggcccttttctttgtgcaatttgagaagggagagagctacttccacatgcacgtgctcgtggaaaccaccggggtgaaatccatggttttgggacgtttcctgagtcagattcgcgaaaaactgattcagagaatttaccgcgggatcgagccgactttgccaaactggttcgcggtcacaaagaccagaaatggcgccggaggcgggaacaaggtggtggatgagtgctacatccccaattacttgctccccaaaacccagcctgagctccagtgggcgtggactaatatggaacagtatttaagcgcctgtttgaatctcacggagcgtaaacggttggtggcgcagcatctgacgcacgtgtcgcagacgcaggagcagaacaaagagaatcagaatcccaattctgatgcgccggtgatcagatcaaaaacttcagccaggtacatggagctggtcgggtggctcgtggacaaggggattacctcggagaagcagtggatccaggaggaccaggcctcatacatctccttcaatgcggcctccaactcgcggtcccaaatcaaggctgccttggacaatgcgggaaagattatgagcctgactaaaaccgcccccgactacctggtgggccagcagcccgtggaggacatttccagcaatcggatttataaaattttggaactaaacgggtacgatccccaatatgcggcttccgtctttctgggatgggccacgaaaaagttcggcaagaggaacaccatctggctgtttgggcctgcaactaccgggaagaccaacatcgcggaggccatagcccacactgtgcccttctacgggtgcgtaaactggaccaatgagaactttcccttcaacgactgtgtcgacaagatggtgatctggtgggaggaggggaagatgaccgccaaggtcgtggagtcggccaaagccattctcggaggaagcaaggtgcgcgtggaccagaaatgcaagtcctcggcccagatagacccgactcccgtgatcgtcacctccaacaccaacatgtgcgccgtgattgacgggaactcaacgaccttcgaacaccagcagccgttgcaagaccggatgttcaaatttgaactcacccgccgtctggatcatgactttgggaaggtcaccaagcaggaagtcaaagactttttccggtgggcaaaggatcacgtggttgaggtggagcatgaattctacgtcaaaaagggtggagccaagaaaagacccgcccccagtgacgcagatataagtgagcccaaacgggtgcgcgagtcagttgcgcagccatcgacgtcagacgcggaagcttcgatcaactacgcagacaggtaccaaaacaaatgttctcgtcacgtgggcatgaatctgatgctgtttccctgcagacaatgcgagagaatgaatcagaattcaaatatctgcttcactcacggacagaaagactgtttagagtgctttcccgtgtcagaatctcaacccgtttctgtcgtcaaaaaggcgtatcagaaactgtgctacattcatcatatcatgggaaaggtgccagacgcttgcactgcctgcgatctggtcaatgtggatttggatgactgcatctttgaacaataaatgatttaaatcaggtatggctgccgatggttatcttccagattggctcgaggacaaccttagtgaaggaattcgcgagtggtgggctttgaaacctggagcccctcaacccaaggcaaatcaacaacatcaagacaacgctcgaggtcttgtgcttccgggttacaaataccttggacccggcaacggactcgacaagggggagccggtcaacgcagcagacgcggcggccctcgagcacgacaaggcctacgaccagcagctcaaggccggagacaacccgtacctcaagtacaaccacgccgacgccgagttccaggagcggctcaaagaagatacgtcttttgggggcaacctcgggcgagcagtcttccaggccaaaaagaggcttcttgaacctcttggtctggttgaggaagcggctaagacggctcctggaaagaagaggcctgtagagcagtctcctcaggaaccggactcctccgcgggtattggcaaatcgggtgcacagcccgctaaaaagagactcaatttcggtcagactggcgacacagagtcagtcccagaccctcaaccaatcggagaacctcccgcagccccctcaggtgtgggatctcttacaatggcttcaggtggtggcgcaccagtggcagacaataacgaaggtgccgatggagtgggtagttcctcgggaaattggcattgcgattcccaatggctgggggacagagtcatcaccaccagcacccgaacctgggccctgcccacctacaacaatcacctctacaagcaaatctccaacagcacatctggaggatcttcaaatgacaacgcctacttcggctacagcaccccctgggggtattttgacttcaacagattccactgccacttctcaccacgtgactggcagcgactcatcaacaacaactggggattccggcctaagcgactcaacttcaagctcttcaacattcaggtcaaagaggttacggacaacaatggagtcaagaccatcgccaataaccttaccagcacggtccaggtcttcacggactcagactatcagctcccgtacgtgctcgggtcggctcacgagggctgcctcccgccgttcccagcggacgttttcatgattcctcagtacgggtatctgacgcttaatgatggaagccaggccgtgggtcgttcgtccttttactgcctggaatatttcccgtcgcaaatgctaagaacgggtaacaacttccagttcagctacgagtttgagaacgtacctttccatagcagctacgctcacagccaaagcctggaccgactaatgaatccactcatcgaccaatacttgtactatctctcaaagactattaacggttctggacagaatcaacaaacgctaaaattcagtgtggccggacccagcaacatggctgtccagggaagaaactacatacctggacccagctaccgacaacaacgtgtctcaaccactgtgactcaaaacaacaacagcgaatttgcttggcctggagcttcttcttgggctctcaatggacgtaatagcttgatgaatcctggacctgctatggccagccacaaagaaggagaggaccgtttctttcctttgtctggatctttaatttttggcaaacaaggaactggaagagacaacgtggatgcggacaaagtcatgataaccaacgaagaagaaattaaaactactaacccggtagcaacggagtcctatggacaagtggccacaaaccaccagagtgcccaagcacaggcgcagaccggctgggttcaaaaccaaggaatacttccgggtatggtttggcaggacagagatgtgtacctgcaaggacccatttgggccaaaattcctcacacggacggcaactttcacccttctccgctgatgggagggtttggaatgaagcacccgcctcctcagatcctcatcaaaaacacacctgtacctgcggatcctccaacggccttcaacaaggacaagctgaactctttcatcacccagtattctactggccaagtcagcgtggagatcgagtgggagctgcagaaggaaaacagcaagcgctggaacccggagatccagtacacttccaactattacaagtctaataatgttgaatttgctgttaatactgaaggtgtatatagtgaaccccgccccattggcaccagatacctgactcgtaatctgtaattgcttgttaatcaataaaccgtttaattcgtttcagttgaactttggtctctgcgtatttctttcttatctagtttccatggctactaaatggcccgcctggctgaccgcccaacgacccccgcccattgacgtcaataatgacgtatgttcccatagtaacgccaatagggactttccattgacgtcaatgggtggagtatttacggtaaactgcccacttggcagtacatcaagtgtatcatatgccaagtacgccccctattgacgtcaatgacggtaaatggcccgcctggcattatgcccagtacatgaccttatgggactttcctacttggcagtacatctacgtattagtcatcgctattaccatggtgatgcggttttggcagtacatcaatgggcgtggatagcggtttgactcacggggatttccaagtctccaccccattgacgtcaatgggagtttgttttggcaccaaaatcaacgggactttccaaaatgtcgtaacaactccgccccattgacgcaaatgggcggtaggcgtgtacggtgggaggtctatataagcagagctggtttagtgaaccggatcctgccattgcatccttctctgcagactaagatggagttcctgaaccaagaccgcttgctggccaacctgtgaaactgggctcaaggtgaggggtgctatctgtgattgagggacatggttaatggaattgtctcacacagaaatcgcacccgtcaccttggcctacttatcaccaccccaaacagaggaacacgccttctccagccacagcctatggaagggccttcagctgctgtggccccgaggtaagcttgggggaggctaactgaaacacggaaggagacaataccggaaggaacccgcgctatgacggcaataaaaagacagaataaaacgcacggtgttgggtcgttgtagataagtagcatggcgggttaatcattaactacagcccgggcgtttaaacagcgggcggaggggtggagtcgtgacgtgaattacgtcatagggttagggaggtcctgtattagaggtcacgtgagtgttttgcgacattttgcgacaccatgtggtctcgctgggggggggggcccgagtgagcacgcagggtctccattttgaagcgggaggtttgaacgagcgctggcgcgctcactggccgtcgttttacaacgtcgtgactgggaaaaccctggcgttacccaacttaatcgccttgcagcacatccccctttcgccagctggcgtaatagcgaagaggcccgcaccgatcgcccttcccaacagttgcgcagcctgaatggcgaatggaaattgtaagcgttaatattttgttaaaattcgcgttaaatttttgttaaatcagctcatttttttaaccaataggccgaaatcggcaaaatcccttataaatcaaaagaatagaccgagatagggttgagtgttgttccagtttggaacaagagtccactattaagaacgtggactccaacgtcaaagggcgaaaaaccgtctatcagggcgatggcccactacgtgaaccatcaccctaatcaagttttttggggtcgaggtgccgtaaagcactaaatcggaaccctaaagggagcccccgatttagagcttgacggggaaagccggcgaacgtggcgagaaaggaagggaagaaagcgaaaggagcgggcgctagggcgctggcaagtgtagcggtcacgctgcgcgtaaccaccacacccgccgcgcttaatgcgccgctacagggcgcgtcaggtggcacttttcggggaaatgtgcgcggaacccctatttgtttatttttctaaatacattcaaatatgtatccgctcatgagacaataaccctgataaatgcttcaataatattgaaaaaggaagagtatgagtattcaacatttccgtgtcgcccttattcccttttttgcggcattttgccttcctgtttttgctcacccagaaacgctggtgaaagtaaaagatgctgaagatcagttgggtgcacgagtgggttacatcgaactggatctcaacagcggtaagatccttgagagttttcgccccgaagaacgttttccaatgatgagcacttttaaagttctgctatgtggcgcggtattatcccgtattgacgccgggcaagagcaactcggtcgccgcatacactattctcagaatgacttggttgagtactcaccagtcacagaaaagcatcttacggatggcatgacagtaagagaattatgcagtgctgccataaccatgagtgataacactgcggccaacttacttctgacaacgatcggaggaccgaaggagctaaccgcttttttgcacaacatgggggatcatgtaactcgccttgatcgttgggaaccggagctgaatgaagccataccaaacgacgagcgtgacaccacgatgcctgtagcaatggcaacaacgttgcgcaaactattaactggcgaactacttactctagcttcccggcaacaattaatagactggatggaggcggataaagttgcaggaccacttctgcgctcggcccttccggctggctggtttattgctgataaatctggagccggtgagcgtgggtctcgcggtatcattgcagcactggggccagatggtaagccctcccgtatcgtagttatctacacgacggggagtcaggcaactatggatgaacgaaatagacagatcgctgagataggtgcctcactgattaagcattggtaactgtcagaccaagtttactcatatatactttagattgatttaaaacttcatttttaatttaaaaggatctaggtgaagatcctttttgataatctcatgaccaaaatcccttaacgtgagttttcgttccactgagcgtcagaccccgtagaaaagatcaaaggatcttcttgagatcctttttttctgcgcgtaatctgctgcttgcaaacaaaaaaaccaccgctaccagcggtggtttgtttgccggatcaagagctaccaactctttttccgaaggtaactggcttcagcagagcgcagataccaaatactgttcttctagtgtagccgtagttaggccaccacttcaagaactctgtagcaccgcctacatacctcgctctgctaatcctgttaccagtggctgctgccagtggcgataagtcgtgtcttaccgggttggactcaagacgatagttaccggataaggcgcagcggtcgggctgaacggggggttcgtgcacacagcccagcttggagcgaacgacctacaccgaactgagatacctacagcgtgagctatgagaaagcgccacgcttcccgaagggagaaaggcggacaggtatccggtaagcggcagggtcggaacaggagagcgcacgagggagcttccagggggaaacgcctggtatctttatagtcctgtcgggtttcgccacctctgacttgagcgtcgatttttgtgatgctcgtcaggggggcggagcctatggaaaaacgccagcaacgcggcctttttacggttcctggccttttgctggccttttgctcacatgttctttcctgcgttatcccctgattctgtggataaccgtattaccgcctttgagtgagctgataccgctcgccgcagccgaacgaccgagcgcagcgagtcagtgagcgaggaagcggaagagcgcccaatacgcaaaccgcctctccccgcgcgttggccgattcattaatgcagctggcacgacaggtttcccgactggaaagcgggcagtgagcgcaacgcaattaatgtgagttagctcactcattaggcaccccaggctttacactttatgcttccggctcgtatgttgtgtggaattgtgagcggataacaatttcacacaggaaacagctatgaccatgattacgccaa

SEQ ID NO: 13 - RNA, 1310 nt, Homo sapiens; identical to SEQ ID NO: 11
  source 1..1310: mol_type = mRNA
  misc_feature 1..1310: note = human NeuroD1 mRNA sequence (ND1-2) comprising modified nucleosides
  modified_base 6..1223: mod_base = m1f; note = Symbol "t" denotes 1-methylpseudouridine, throughout the sequence

SEQ ID NO: 14 - DNA, 1672 bp, Homo sapiens
  source 1..1672: mol_type = genomic DNA
  misc_feature 1..1672: note = human GFAP promoter
gtctgcaagcagacctggcagcattgggctggccgccccccagggcctcctcttcatgcccagtgaatgactcaccttggcacagacacaatgttcggggtgggcacagtgcctgcttcccgccgcaccccagcccccctcaaatgccttccgagaagcccattgagtagggggcttgcattgcaccccagcctgacagcctggcatcttgggataaaagcagcacagccccctaggggctgcccttgctgtgtggcgccaccggcggtggagaacaaggctctattcagcctgtgcccaggaaaggggatcaggggatgcccaggcatggacagtgggtggcagggggggagaggagggctgtctgcttcccagaagtccaaggacacaaatgggtgaggggactgggcagggttctgaccctgtgggaccagagtggagggcgtagatggacctgaagtctccagggacaacagggcccaggtctcaggctcctagttgggcccagtggctccagcgtttccaaacccatccatccccagaggttcttcccatctctccaggctgatgtgtgggaactcgaggaaataaatctccagtgggagacggaggggtggccagggaaacggggcgctgcaggaataaagacgagccagcacagccagctcatgcgtaacggctttgtggagctgtcaaggcctggtctctgggagagaggcacagggaggccagacaaggaaggggtgacctggagggacagatccaggggctaaagtcctgataaggcaagagagtgccggccccctcttgccctatcaggacctccactgccacatagaggccatgattgacccttagacaaagggctggtgtccaatcccagcccccagccccagaactccagggaatgaatgggcagagagcaggaatgtgggacatctgtgttcaagggaaggactccaggagtctgctgggaatgaggcctagtaggaaatgaggtggcccttgagggtacagaacaggttcattcttcgccaaattcccagcaccttgcaggcacttacagctgagtgagataatgcctgggttatgaaatcaaaaagttggaaagcaggtcagaggtcatctggtacagcccttccttccctttttttttttttttttttgtgagacaaggtctctctctgttgcccaggctggagtggcgcaaacacagctcactgcagcctcaacctactgggctcaagcaatcctccagcctcagcctcccaaagtgctgggattacaagcatgagccaccccactcagccctttccttcctttttaattgatgcataataattgtaagtattcatcatggtccaaccaaccctttcttgacccaccttcctagagagagggtcctcttgattcagcggtcagggccccagacccatggtctggctccaggtaccacctgcctcatgcaggagttggcgtgcccaggaagctctgcctctgggcacagtgacctcagtggggtgaggggagctctccccatagctgggctgcggcccaaccccaccccctcaggctatgccagggggtgttgccaggggcacccgggcatcgccagtctagcccactccttcataaagccctcgcatcccaggagcgagcagagccagagcat